European Patent Application EP 4 368 636 A1, published May 15, 2024. Title: 融合蛋白及其应用. Applicant: 苏州康宁杰瑞生物科技有限公司. The sequence listing filed with the application follows.

SEQUENCE LISTING (84 sequences)

SEQ ID NO: 1 - protein, 31 aa, synthetic construct
  REGION 1..31: note = GLP-1wt
HAEGTFTSDVSSYLEGQAAKEFIAWLVKGRG

SEQ ID NO: 2 - protein, 31 aa, synthetic construct
  REGION 1..31: note = GLP-1/dulaglutide
HGEGTFTSDVSSYLEEQAAKEFIAWLVKGGG

SEQ ID NO: 3 - protein, 275 aa, synthetic construct
  REGION 1..275: note = dulaglutide/DULA
HGEGTFTSDVSSYLEEQAAKEFIAWLVKGGGGGGGSGGGGSGGGGSAESKYGPPCPPCPAPEAAGGPSVFLFPPKPKDTLMISRTPEVTCVVVDVSQEDPEVQFNWYVDGVEVHNAKTKPREEQFNSTYRVVSVLTVLHQDWLNGKEYKCKVSNKGLPSSIEKTISKAKGQPREPQVYTLPPSQEEMTKNQVSLTCLVKGFYPSDIAVEWESNGQPENNYKTTPPVLDSDGSFFLYSRLTVDKSRWQEGNVFSCSVMHEALHNHYTQKSLSLSLG

SEQ ID NO: 4 - protein, 31 aa, synthetic construct
  REGION 1..31: note = GLP-1-KRWY
HGEGTFTSDVSSYLEEQAAREFIAYLVKGGG

SEQ ID NO: 5 - protein, 31 aa, synthetic construct
  REGION 1..31: note = GLP-1-KRYL
HGEGTFTSDVSSLLEEQAAREFIAWLVKGGG

SEQ ID NO: 6 - protein, 31 aa, synthetic construct
  REGION 1..31: note = GLP-1-KRYT
HGEGTFTSDVSSTLEEQAAREFIAWLVKGGG

SEQ ID NO: 7 - protein, 31 aa, synthetic construct
  REGION 1..31: note = GLP-1-KRYF
HGEGTFTSDVSSFLEEQAAREFIAWLVKGGG

SEQ ID NO: 8 - protein, 31 aa, synthetic construct
  REGION 1..31: note = GLP-1-KRYI
HGEGTFTSDVSSILEEQAAREFIAWLVKGGG

SEQ ID NO: 9 - protein, 31 aa, synthetic construct
  REGION 1..31: note = GLP-1-KRYV
HGEGTFTSDVSSVLEEQAAREFIAWLVKGGG

SEQ ID NO: 10 - protein, 31 aa, synthetic construct
  REGION 1..31: note = GLP-1-KRYS
HGEGTFTSDVSSSLEEQAAREFIAWLVKGGG

SEQ ID NO: 11 - protein, 31 aa, synthetic construct
  REGION 1..31: note = GLP-1-KRYA
HGEGTFTSDVSSALEEQAAREFIAWLVKGGG

SEQ ID NO: 12 - protein, 31 aa, synthetic construct
  REGION 1..31: note = GLP-1-WYYL
HGEGTFTSDVSSLLEEQAAKEFIAYLVKGGG

SEQ ID NO: 13 - protein, 31 aa, synthetic construct
  REGION 1..31: note = GLP-1-WYYT
HGEGTFTSDVSSTLEEQAAKEFIAYLVKGGG

SEQ ID NO: 14 - protein, 31 aa, synthetic construct
  REGION 1..31: note = GLP-1-WYYF
HGEGTFTSDVSSFLEEQAAKEFIAYLVKGGG

SEQ ID NO: 15 - protein, 31 aa, synthetic construct
  REGION 1..31: note = GLP-1-WYYI
HGEGTFTSDVSSILEEQAAKEFIAYLVKGGG

SEQ ID NO: 16 - protein, 31 aa, synthetic construct
  REGION 1..31: note = GLP-1-WYYV
HGEGTFTSDVSSVLEEQAAKEFIAYLVKGGG

SEQ ID NO: 17 - protein, 31 aa, synthetic construct
  REGION 1..31: note = GLP-1-WYYS
HGEGTFTSDVSSSLEEQAAKEFIAYLVKGGG

SEQ ID NO: 18 - protein, 31 aa, synthetic construct
  REGION 1..31: note = GLP-1-WYYA
HGEGTFTSDVSSALEEQAAKEFIAYLVKGGG

SEQ ID NO: 19 - protein, 31 aa, synthetic construct
  REGION 1..31: note = GLP-1-KRWYYF
HGEGTFTSDVSSFLEEQAAREFIAYLVKGGG

SEQ ID NO: 20 - protein, 31 aa, synthetic construct
  REGION 1..31: note = GLP-1-KRWYYL
HGEGTFTSDVSSLLEEQAAREFIAYLVKGGG

SEQ ID NO: 21 - protein, 31 aa, synthetic construct
  REGION 1..31: note = GLP-1-KRWYYT
HGEGTFTSDVSSTLEEQAAREFIAYLVKGGG

SEQ ID NO: 22 - protein, 31 aa, synthetic construct
  REGION 1..31: note = GLP-1-KRWYYI
HGEGTFTSDVSSILEEQAAREFIAYLVKGGG

SEQ ID NO: 23 - protein, 31 aa, synthetic construct
  REGION 1..31: note = GLP-1-KRWYYV
HGEGTFTSDVSSVLEEQAAREFIAYLVKGGG

SEQ ID NO: 24 - protein, 31 aa, synthetic construct
  REGION 1..31: note = GLP-1-KRWYYS
HGEGTFTSDVSSSLEEQAAREFIAYLVKGGG

SEQ ID NO: 25 - protein, 31 aa, synthetic construct
  REGION 1..31: note = GLP-1-KRWYYA
HGEGTFTSDVSSALEEQAAREFIAYLVKGGG

SEQ ID NO: 26 - protein, 31 aa, synthetic construct
  REGION 1..31: note = GLP-1 formula
  SITE 13: note = misc_feature - Xaa = Ala, Phe, Ile, Leu, Ser, Thr, Val or Tyr
  SITE 25: note = misc_feature - Xaa = Ala, Lys, Arg, Trp or Tyr
HGEGTFTSDVSSXLEEQAAREFIAXLVKGGG

SEQ ID NO: 27 - protein, 15 aa, synthetic construct
  REGION 1..15: note = L1
GGGGSGGGGSGGGGS

SEQ ID NO: 28 - protein, 15 aa, synthetic construct
  REGION 1..15: note = L2
ASTKGPSVFPLAGGG

SEQ ID NO: 29 - protein, 15 aa, synthetic construct
  REGION 1..15: note = L3
GGGGGGGGGGGGGGG

SEQ ID NO: 30 - protein, 15 aa, synthetic construct
  REGION 1..15: note = H1
EPKSSDKTHTCPPCP

SEQ ID NO: 31 - protein, 13 aa, synthetic construct
  REGION 1..13: note = H2
AESKYGPPCPPCP

SEQ ID NO: 32 - protein, 217 aa, synthetic construct
  REGION 1..217: note = Fc1
APELLGGPSVFLFPPKPKDTLMISRTPEVTCVVVDVSHEDPEVKFNWYVDGVEVHNAKTKPREEQYNSTYRVVSVLTVLHQDWLNGKEYKCKVSNKALPAPIEKTISKAKGQPREPQVYTLPPSRDELTKNQVSLTCLVKGFYPSDIAVEWESNGQPENNYKTTPPVLDSDGSFFLYSKLTVDKSRWQQGNVFSCSVMHEALHNHYTQKSLSLSPGK

SEQ ID NO: 33 - protein, 216 aa, synthetic construct
  REGION 1..216: note = Fc2
APPVAGPSVFLFPPKPKDTLMISRTPEVTCVVVDVSHEDPEVQFNWYVDGVEVHNAKTKPREEQFNSTFRVVSVLTVVHQDWLNGKEYKCKVSNKGLPAPIEKTISKTKGQPREPQVYTLPPSREEMTKNQVSLTCLVKGFYPSDISVEWESNGQPENNYKTTPPMLDSDGSFFLYSKLTVDKSRWQQGNVFSCSVMHEALHNHYTQKSLSLSPGK

SEQ ID NO: 34 - protein, 217 aa, synthetic construct
  REGION 1..217: note = Fc3
APELLGGPSVFLFPPKPKDTLMISRTPEVTCVVVDVSHEDPEVQFKWYVDGVEVHNAKTKPREEQYNSTFRVVSVLTVLHQDWLNGKEYKCKVSNKALPAPIEKTISKTKGQPREPQVYTLPPSREEMTKNQVSLTCLVKGFYPSDIAVEWESSGQPENNYNTTPPMLDSDGSFFLYSKLTVDKSRWQQGNIFSCSVMHEALHNRFTQKSLSLSPGK

SEQ ID NO: 35 - protein, 217 aa, synthetic construct
  REGION 1..217: note = Fc4
APEFLGGPSVFLFPPKPKDTLMISRTPEVTCVVVDVSQEDPEVQFNWYVDGVEVHNAKTKPREEQFNSTYRVVSVLTVLHQDWLNGKEYKCKVSNKGLPSSIEKTISKAKGQPREPQVYTLPPSQEEMTKNQVSLTCLVKGFYPSDIAVEWESNGQPENNYKTTPPVLDSDGSFFLYSRLTVDKSRWQEGNVFSCSVMHEALHNHYTQKSLSLSLGK

SEQ ID NO: 36 - protein, 217 aa, synthetic construct
  REGION 1..217: note = Fc4m
APEFLGGPSVFLFPPKPKDTLYITREPEVTCVVVDVSQEDPEVQFNWYVDGVEVHNAKTKPREEQFNSTYRVVSVLTVLHQDWLNGKEYKCKVSNKGLPSSIEKTISKAKGQPREPQVYTLPPSQEEMTKNQVSLTCLVKGFYPSDIAVEWESNGQPENNYKTTPPVLDSDGSFFLYSRLTVDKSRWQEGNVFSCSVMHEALHNHYTQKSLSLSLGK

SEQ ID NO: 37 - protein, 275 aa, synthetic construct
  REGION 1..275: note = GM-RY-L1H2-Fc4
HGEGTFTSDVSSYLEEQAAREFIAYLVKGGGGGGGSGGGGSGGGGSAESKYGPPCPPCPAPEFLGGPSVFLFPPKPKDTLMISRTPEVTCVVVDVSQEDPEVQFNWYVDGVEVHNAKTKPREEQFNSTYRVVSVLTVLHQDWLNGKEYKCKVSNKGLPSSIEKTISKAKGQPREPQVYTLPPSQEEMTKNQVSLTCLVKGFYPSDIAVEWESNGQPENNYKTTPPVLDSDGSFFLYSRLTVDKSRWQEGNVFSCSVMHEALHNHYTQKSLSLSLG

SEQ ID NO: 38 - protein, 276 aa, synthetic construct
  REGION 1..276: note = GM-RY-L2H2-Fc4
HGEGTFTSDVSSYLEEQAAREFIAYLVKGGGASTKGPSVFPLAGGGAESKYGPPCPPCPAPEFLGGPSVFLFPPKPKDTLMISRTPEVTCVVVDVSQEDPEVQFNWYVDGVEVHNAKTKPREEQFNSTYRVVSVLTVLHQDWLNGKEYKCKVSNKGLPSSIEKTISKAKGQPREPQVYTLPPSQEEMTKNQVSLTCLVKGFYPSDIAVEWESNGQPENNYKTTPPVLDSDGSFFLYSRLTVDKSRWQEGNVFSCSVMHEALHNHYTQKSLSLSLGK

SEQ ID NO: 39 - protein, 276 aa, synthetic construct
  REGION 1..276: note = GM-RY-L3H2-Fc4
HGEGTFTSDVSSYLEEQAAREFIAYLVKGGGGGGGGGGGGGGGGGGAESKYGPPCPPCPAPEFLGGPSVFLFPPKPKDTLMISRTPEVTCVVVDVSQEDPEVQFNWYVDGVEVHNAKTKPREEQFNSTYRVVSVLTVLHQDWLNGKEYKCKVSNKGLPSSIEKTISKAKGQPREPQVYTLPPSQEEMTKNQVSLTCLVKGFYPSDIAVEWESNGQPENNYKTTPPVLDSDGSFFLYSRLTVDKSRWQEGNVFSCSVMHEALHNHYTQKSLSLSLGK

SEQ ID NO: 40 - protein, 276 aa, synthetic construct
  REGION 1..276: note = GM-ARY-L2H2-Fc4
HGEGTFTSDVSSALEEQAAREFIAYLVKGGGASTKGPSVFPLAGGGAESKYGPPCPPCPAPEFLGGPSVFLFPPKPKDTLMISRTPEVTCVVVDVSQEDPEVQFNWYVDGVEVHNAKTKPREEQFNSTYRVVSVLTVLHQDWLNGKEYKCKVSNKGLPSSIEKTISKAKGQPREPQVYTLPPSQEEMTKNQVSLTCLVKGFYPSDIAVEWESNGQPENNYKTTPPVLDSDGSFFLYSRLTVDKSRWQEGNVFSCSVMHEALHNHYTQKSLSLSLGK

SEQ ID NO: 41 - protein, 278 aa, synthetic construct
  REGION 1..278: note = GM-ARY-L2H1-Fc4
HGEGTFTSDVSSALEEQAAREFIAYLVKGGGASTKGPSVFPLAGGGEPKSSDKTHTCPPCPAPEFLGGPSVFLFPPKPKDTLMISRTPEVTCVVVDVSQEDPEVQFNWYVDGVEVHNAKTKPREEQFNSTYRVVSVLTVLHQDWLNGKEYKCKVSNKGLPSSIEKTISKAKGQPREPQVYTLPPSQEEMTKNQVSLTCLVKGFYPSDIAVEWESNGQPENNYKTTPPVLDSDGSFFLYSRLTVDKSRWQEGNVFSCSVMHEALHNHYTQKSLSLSLGK

SEQ ID NO: 42 - protein, 276 aa, synthetic construct
  REGION 1..276: note = GM-ARY-L2H2-Fc4m
HGEGTFTSDVSSALEEQAAREFIAYLVKGGGASTKGPSVFPLAGGGAESKYGPPCPPCPAPEFLGGPSVFLFPPKPKDTLYITREPEVTCVVVDVSQEDPEVQFNWYVDGVEVHNAKTKPREEQFNSTYRVVSVLTVLHQDWLNGKEYKCKVSNKGLPSSIEKTISKAKGQPREPQVYTLPPSQEEMTKNQVSLTCLVKGFYPSDIAVEWESNGQPENNYKTTPPVLDSDGSFFLYSRLTVDKSRWQEGNVFSCSVMHEALHNHYTQKSLSLSLGK

SEQ ID NO: 43 - protein, 278 aa, synthetic construct
  REGION 1..278: note = GM-RY-L2H1-Fc4m
HGEGTFTSDVSSYLEEQAAREFIAYLVKGGGASTKGPSVFPLAGGGEPKSSDKTHTCPPCPAPEFLGGPSVFLFPPKPKDTLYITREPEVTCVVVDVSQEDPEVQFNWYVDGVEVHNAKTKPREEQFNSTYRVVSVLTVLHQDWLNGKEYKCKVSNKGLPSSIEKTISKAKGQPREPQVYTLPPSQEEMTKNQVSLTCLVKGFYPSDIAVEWESNGQPENNYKTTPPVLDSDGSFFLYSRLTVDKSRWQEGNVFSCSVMHEALHNHYTQKSLSLSLGK

SEQ ID NO: 44 - protein, 278 aa, synthetic construct
  REGION 1..278: note = GM-ARY-L2H1-Fc4m
HGEGTFTSDVSSALEEQAAREFIAYLVKGGGASTKGPSVFPLAGGGEPKSSDKTHTCPPCPAPEFLGGPSVFLFPPKPKDTLYITREPEVTCVVVDVSQEDPEVQFNWYVDGVEVHNAKTKPREEQFNSTYRVVSVLTVLHQDWLNGKEYKCKVSNKGLPSSIEKTISKAKGQPREPQVYTLPPSQEEMTKNQVSLTCLVKGFYPSDIAVEWESNGQPENNYKTTPPVLDSDGSFFLYSRLTVDKSRWQEGNVFSCSVMHEALHNHYTQKSLSLSLGK

SEQ ID NO: 45 - protein, 276 aa, synthetic construct
  REGION 1..276: note = GM-RY-L2H2-Fc4m
HGEGTFTSDVSSYLEEQAAREFIAYLVKGGGASTKGPSVFPLAGGGAESKYGPPCPPCPAPEFLGGPSVFLFPPKPKDTLYITREPEVTCVVVDVSQEDPEVQFNWYVDGVEVHNAKTKPREEQFNSTYRVVSVLTVLHQDWLNGKEYKCKVSNKGLPSSIEKTISKAKGQPREPQVYTLPPSQEEMTKNQVSLTCLVKGFYPSDIAVEWESNGQPENNYKTTPPVLDSDGSFFLYSRLTVDKSRWQEGNVFSCSVMHEALHNHYTQKSLSLSLGK

SEQ ID NO: 46 - protein, 276 aa, synthetic construct
  REGION 1..276: note = DULA-Fc4m
HGEGTFTSDVSSYLEEQAAKEFIAWLVKGGGGGGGSGGGGSGGGGSAESKYGPPCPPCPAPEFLGGPSVFLFPPKPKDTLYITREPEVTCVVVDVSQEDPEVQFNWYVDGVEVHNAKTKPREEQFNSTYRVVSVLTVLHQDWLNGKEYKCKVSNKGLPSSIEKTISKAKGQPREPQVYTLPPSQEEMTKNQVSLTCLVKGFYPSDIAVEWESNGQPENNYKTTPPVLDSDGSFFLYSRLTVDKSRWQEGNVFSCSVMHEALHNHYTQKSLSLSLGK

SEQ ID NO: 47 - protein, 16 aa, synthetic construct
  REGION 1..16: note = L4
AKTTPKLEEGEFSEAR

SEQ ID NO: 48 - protein, 17 aa, synthetic construct
  REGION 1..17: note = L5
AKTTPKLEEGEFSEARV

SEQ ID NO: 49 - protein, 9 aa, synthetic construct
  REGION 1..9: note = L6
AKTTPKLGG

SEQ ID NO: 50 - protein, 10 aa, synthetic construct
  REGION 1..10: note = L7
SAKTTPKLGG

SEQ ID NO: 51 - protein, 6 aa, synthetic construct
  REGION 1..6: note = L8
SAKTTP

SEQ ID NO: 52 - protein, 6 aa, synthetic construct
  REGION 1..6: note = L9
RADAAP

SEQ ID NO: 53 - protein, 9 aa, synthetic construct
  REGION 1..9: note = L10
RADAAPTVS

SEQ ID NO: 54 - protein, 12 aa, synthetic construct
  REGION 1..12: note = L11
RADAAAAGGPGS

SEQ ID NO: 55 - protein, 18 aa, synthetic construct
  REGION 1..18: note = L12
SAKTTPKLEEGEFSEARV

SEQ ID NO: 56 - protein, 5 aa, synthetic construct
  REGION 1..5: note = L13
ADAAP

SEQ ID NO: 57 - protein, 12 aa, synthetic construct
  REGION 1..12: note = L14
ADAAPTVSIFPP

SEQ ID NO: 58 - protein, 5 aa, synthetic construct
  REGION 1..5: note = L15
TVAAP

SEQ ID NO: 59 - protein, 12 aa, synthetic construct
  REGION 1..12: note = L16
TVAAPSVFIFPP

SEQ ID NO: 60 - protein, 6 aa, synthetic construct
  REGION 1..6: note = L17
QPKAAP

SEQ ID NO: 61 - protein, 13 aa, synthetic construct
  REGION 1..13: note = L18
QPKAAPSVTLFPP

SEQ ID NO: 62 - protein, 6 aa, synthetic construct
  REGION 1..6: note = L19
AKTTPP

SEQ ID NO: 63 - protein, 13 aa, synthetic construct
  REGION 1..13: note = L20
AKTTPPSVTPLAP

SEQ ID NO: 64 - protein, 6 aa, synthetic construct
  REGION 1..6: note = L21
AKTTAP

SEQ ID NO: 65 - protein, 13 aa, synthetic construct
  REGION 1..13: note = L22
AKTTAPSVYPLAP

SEQ ID NO: 66 - protein, 6 aa, synthetic construct
  REGION 1..6: note = L23
ASTKGP

SEQ ID NO: 67 - protein, 13 aa, synthetic construct
  REGION 1..13: note = L24
ASTKGPSVFPLAP

SEQ ID NO: 68 - protein, 15 aa, synthetic construct
  REGION 1..15: note = L25
GENKVEYAPALMALS

SEQ ID NO: 69 - protein, 15 aa, synthetic construct
  REGION 1..15: note = L26
GPAKELTPLKEAKVS

SEQ ID NO: 70 - protein, 15 aa, synthetic construct
  REGION 1..15: note = L27
GHEAAAVMQVQYPAS

SEQ ID NO: 71 - protein, 31 aa, synthetic construct
  REGION 1..31: note = GLP-1-WY
HGEGTFTSDVSSYLEEQAAKEFIAYLVKGGG

SEQ ID NO: 72 - protein, 31 aa, synthetic construct
  REGION 1..31: note = GLP-1-KRQN
HGEGTFTSDVSSYLEENAAREFIAWLVKGGG

SEQ ID NO: 73 - protein, 31 aa, synthetic construct
  REGION 1..31: note = GLP-1-KRQT
HGEGTFTSDVSSYLEETAAREFIAWLVKGGG

SEQ ID NO: 74 - protein, 31 aa, synthetic construct
  REGION 1..31: note = GLP-1-KRQS
HGEGTFTSDVSSYLEESAAREFIAWLVKGGG

SEQ ID NO: 75 - protein, 31 aa, synthetic construct
  REGION 1..31: note = GLP-1-KRQE
HGEGTFTSDVSSYLEEEAAREFIAWLVKGGG

SEQ ID NO: 76 - protein, 31 aa, synthetic construct
  REGION 1..31: note = GLP-1-WYQN
HGEGTFTSDVSSYLEENAAKEFIAYLVKGGG

SEQ ID NO: 77 - protein, 31 aa, synthetic construct
  REGION 1..31: note = GLP-1-WYQS
HGEGTFTSDVSSYLEESAAKEFIAYLVKGGG

SEQ ID NO: 78 - protein, 31 aa, synthetic construct
  REGION 1..31: note = GLP-1-WYQT
HGEGTFTSDVSSYLEETAAKEFIAYLVKGGG

SEQ ID NO: 79 - protein, 31 aa, synthetic construct
  REGION 1..31: note = GLP-1-WYQE
HGEGTFTSDVSSYLEEEAAKEFIAYLVKGGG

SEQ ID NO: 80 - protein, 31 aa, synthetic construct
  REGION 1..31: note = GLP-1-WYFL
HGEGTFTSDVSSYLEEQAAKELIAYLVKGGG

SEQ ID NO: 81 - protein, 31 aa, synthetic construct
  REGION 1..31: note = GLP-1-KRWYQN
HGEGTFTSDVSSYLEENAAREFIAYLVKGGG

SEQ ID NO: 82 - protein, 31 aa, synthetic construct
  REGION 1..31: note = GLP-1-KRWYQT
HGEGTFTSDVSSYLEETAAREFIAYLVKGGG

SEQ ID NO: 83 - protein, 31 aa, synthetic construct
  REGION 1..31: note = GLP-1-KRWYQS
HGEGTFTSDVSSYLEESAAREFIAYLVKGGG

SEQ ID NO: 84 - protein, 31 aa, synthetic construct
  REGION 1..31: note = GLP-1-KRWYQE
HGEGTFTSDVSSYLEEEAAREFIAYLVKGGG